European Patent Specification EP 3 313 876 B1, published January 22, 2025. Title: MULTISPECIFIC ANTIGEN BINDING PROTEINS. Applicant: INNATE PHARMA. The sequence listing filed with the application follows.

SEQUENCE LISTING (78 sequences)

SEQ ID NO: 1 - protein, 216 aa, Homo sapiens
APELLGGPSVFLFPPKPKDTLMISRTPEVTCVVVDVSHEDPEVKFNWYVDGVEVHNAKTKPREEQYNSTYRVVSVLTVLHQDWLNGKEYKCKVSNKALPAPIEKTISKAKGQPREPQVYTLPPSREEMTKNQVSLTCLVKGFYPSDIAVEWESNGQPENNYKTTPPVLDSDGSFFLTSKLTVDKSRWQQGNVFSCSVMHEALHNHYTQKSLSLSPG

SEQ ID NO: 2 - protein, 227 aa, Homo sapiens
GQPREPQVYTLPPSREEMTKNQVSLTCLVKGFYPSDIAVEWESNGQPENNYKTTPPVLDSDGSFFLYSKLTVDKSRWQQGNVFSCSVMHEALHNHYTQKSLSLSPGGGGGSGGGGSGGGGSGQPREPQVYTLPPSREEMTKNQVSLTCLVKGFYPSDIAVEWESNGQPENNYKTTPPVLDSDGSFFLYSKLTVDKSRWQQGNVFSCSVMHEALHNHYTQKSLSLSPG

SEQ ID NO: 3 - DNA, 333 bp, mus musculus
gacattcagctgacccaatctccagcttctttggctgtgtctctagggcagagggccaccatctcctgcaaggccagccaaagtgttgattatgatggtgatagttatttgaactggtaccaacagataccaggacagccacccaaactcctcatctatgatgcatccaatctagtatctgggattccacccaggtttagtggcagtgggtctgggacagacttcaccctcaacatccatcctgtggagaaggtggatgctgcaacctatcactgtcagcaaagtactgaggacccttggacgttcggtggaggcaccaagctggaaatcaaa

SEQ ID NO: 4 - protein, 111 aa, mus musculus
DIQLTQSPASLAVSLGQRATISCKASQSVDYDGDSYLNWYQQIPGQPPKLLIYDASNLVSGIPPRFSGSGSGTDFTLNIHPVEKVDAATYHCQQSTEDPWTFGGGTKLEIK

SEQ ID NO: 5 - DNA, 372 bp, mus musculus
caggttcagctgcagcagtctggggctgagctggtgcggcctgggtcctcagtgaagatttcctgcaaagcatctggctacgcattcagtagctactggatgaactgggtgaagcagaggcctggacagggtcttgagtggattggacagatttggcctggagatggtgatactaactacaacggaaagttcaagggcaaggccacactgactgcagacgaatcctccagcacagcctacatgcagctcagcagcctggcctctgaggactctgcggtctatttctgtgcaagacgagaaacgaccactgtcgggcgttattactatgctatggactactggggtcaaggaaccacagtcaccgtctcctca

SEQ ID NO: 6 - protein, 124 aa, mus musculus
QVQLQQSGAELVRPGSSVKISCKASGYAFSSYWMNWVKQRPGQGLEWIGQIWPGDGDTNYNGKFKGKATLTADESSSTAYMQLSSLASEDSAVYFCARRETTTVGRYYYAMDYWGQGTTVTVSS

SEQ ID NO: 7 - DNA, 648 bp, homo sapiens
gcacctgaactcctggggggaccgtcagtcttcctcttccccccaaaacccaaggacaccctcatgatctcccggacccctgaggtcacatgcgtggtggtggacgtgagccacgaagaccctgaggtcaagttcaactggtacgtggacggcgtggaggtgcataatgccaagacaaagccgcgggaggagcagtacaacagcacgtaccgtgtggtcagcgtcctcaccgtcctgcaccaggactggctgaatggcaaggagtacaagtgcaaggtctccaacaaagccctcccagcccccatcgagaaaaccatctccaaagccaaagggcagccccgagaaccacaggtgtacaccaagcccccatcccgggaggagatgaccaagaaccaggtcagcctgtcctgcctggtcaaaggcttctatcccagcgacatcgccgtggagtgggagagcaatgggcagccggagaacaactacaagaccacggttcccgtgctggactccgacggctccttccgcctcgctagctacctcaccgtggacaagagcaggtggcagcaggggaacgtcttctcatgctccgtgatgcatgaggctctgcacaaccactacacgcagaagagcctctccctgtccccgggg

SEQ ID NO: 8 - protein, 216 aa, homo sapiens
APELLGGPSVFLFPPKPKDTLMISRTPEVTCVVVDVSHEDPEVKFNWYVDGVEVHNAKTKPREEQYNSTYRVVSVLTVLHQDWLNGKEYKCKVSNKALPAPIEKTISKAKGQPREPQVYTKPPSREEMTKNQVSLSCLVKGFYPSDIAVEWESNGQPENNYKTTVPVLDSDGSFRLASYLTVDKSRWQQGNVFSCSVMHEALHNHYTQKSLSLSPG

SEQ ID NO: 9 - protein, 718 aa, Artificial
  Chimeric homo sapiens-mus musculus
DIQLTQSPASLAVSLGQRATISCKASQSVDYDGDSYLNWYQQIPGQPPKLLIYDASNLVSGIPPRFSGSGSGTDFTLNIHPVEKVDAATYHCQQSTEDPWTFGGGTKLEIKGGGGSGGGGSGGGGSQVQLQQSGAELVRPGSSVKISCKASGYAFSSYWMNWVKQRPGQGLEWIGQIWPGDGDTNYNGKFKGKATLTADESSSTAYMQLSSLASEDSAVYFCARRETTTVGRYYYAMDYWGQGTTVTVSSGGGSSAPELLGGPSVFLFPPKPKDTLMISRTPEVTCVVVDVSHEDPEVKFNWYVDGVEVHNAKTKPREEQYNSTYRVVSVLTVLHQDWLNGKEYKCKVSNKALPAPIEKTISKAKGQPREPQVYTKPPSREEMTKNQVSLSCLVKGFYPSDIAVEWESNGQPENNYKTTVPVLDSDGSFRLASYLTVDKSRWQQGNVFSCSVMHEALHNHYTQKSLSLSPGSTGSDIKLQQSGAELARPGASVKMSCKTSGYTFTRYTMHWVKQRPGQGLEWIGYINPSRGYTNYNQKFKDKATLTTDKSSSTAYMQLSSLTSEDSAVYYCARYYDDHYCLDYWGQGTTLTVSSVEGGSGGSGGSGGSGGVDDIQLTQSPAIMSASPGEKVTMTCRASSSVSYMNWYQQKSGTSPKRWIYDTSKVASGVPYRFSGSGSGTSYSLTISSMEAEDAATYYCQQWSSNPLTFGAGTKLELK

SEQ ID NO: 10 - protein, 245 aa, Mus musculus
STGSEVQLQQSGPELVKPGASVKISCKTSGYTFTEYTMHWVKQSHGKSLEWIGGISPNIGGTSYNQKFKGKATLTVDKSSSTAYMELRSLTSEDSAVYYCARRGGSFDYWGQGTTLTVSSVEGGSGGSGGSGGSGGVDDIVMTQSPATLSVTPGDRVSLSCRASQSISDYLHWYQQKSHESPRLLIKYASQSISGIPSRFSGSGSGSDFTLSINSVEPEDVGVYYCQNGHSFPLTFGAGTKLELK

SEQ ID NO: 11 - protein, 698 aa, Artificial
  Chimeric homo sapiens - mus musculus
DIQLTQSPASLAVSLGQRATISCKASQSVDYDGDSYLNWYQQIPGQPPKLLIYDASNLVSGIPPRFSGSGSGTDFTLNIHPVEKVDAATYHCQQSTEDPWTFGGGTKLEIKGGGGSGGGGSGGGGSQVQLQQSGAELVRPGSSVKISCKASGYAFSSYWMNWVKQRPGQGLEWIGQIWPGDGDTNYNGKFKGKATLTADESSSTAYMQLSSLASEDSAVYFCARRETTTVGRYYYAMDYWGQGTTVTVSSGGGSSAPELLGGPSVFLFPPKPKDTLMISRTPEVTCVVVDVSHEDPEVKFNWYVDGVEVHNAKTKPREEQYNSTYRVVSVLTVLHQDWLNGKEYKCKVSNKALPAPIEKTISKAKGQPREPQVYTKPPSREEMTKNQVSLSCLVKGFYPSDIAVEWESNGQPENNYKTTVPVLDSDGSFRLASYLTVDKSRWQQGNVFSCSVMHEALHNHYTQKSLSLSPGSTGSEVQLQQSGPELVKPGASVKISCKTSGYTFTEYTMHWVKQSHGKSLEWIGGISPNIGGTSYNQKFKGKATLTVDKSSSTAYMELRSLTSEDSAVYYCARRGGSFDYWGQGTTLTVSSASTKGPSVFPLAPSSKSTSGGTAALGCLVKDYFPEPVTVSWNSGALTSGVHTFPAVLQSSGLYSLSSVVTVPSSSLGTQTYICNVNHKPSNTKVDKRVEPKSCDKTH

SEQ ID NO: 12 - protein, 214 aa, Artificial
  Chimeric - homo sapiens mus musculus
DIVMTQSPATLSVTPGDRVSLSCRASQSISDYLHWYQQKSHESPRLLIKYASQSISGIPSRFSGSGSGSDFTLSINSVEPEDVGVYYCQNGHSFPLTFGAGTKLELKRTVAAPSVFIFPPSDEQLKSGTASVVCLLNNFYPREAKVQWKVDNALQSGNSQESVTEQDSKDSTYSLSSTLTLSKADYEKHKVYACEVTHQGLSSPVTKSFNRGEC

SEQ ID NO: 13 - protein, 218 aa, Artificial
  Chimeric homo sapiens mus musculus
DIQLTQSPASLAVSLGQRATISCKASQSVDYDGDSYLNWYQQIPGQPPKLLIYDASNLVSGIPPRFSGSGSGTDFTLNIHPVEKVDAATYHCQQSTEDPWTFGGGTKLEIKRTVAAPSVFIFPPSDEQLKSGTASVVCLLNNFYPREAKVQWKVDNALQSGNSQESVTEQDSKDSTYSLSSTLTLSKADYEKHKVYACEVTHQGLSSPVTKSFNRGEC

SEQ ID NO: 14 - protein, 675 aa, Artificial
  Chimeric homo sapiens mus musculus
QVQLQQSGAELVRPGSSVKISCKASGYAFSSYWMNWVKQRPGQGLEWIGQIWPGDGDTNYNGKFKGKATLTADESSSTAYMQLSSLASEDSAVYFCARRETTTVGRYYYAMDYWGQGTTVTVSSASTKGPSVFPLAPSSKSTSGGTAALGCLVKDYFPEPVTVSWNSGALTSGVHTFPAVLQSSGLYSLSSVVTVPSSSLGTQTYICNVNHKPSNTKVDKRVEPKSCGGGSSAPELLGGPSVFLFPPKPKDTLMISRTPEVTCVVVDVSHEDPEVKFNWYVDGVEVHNAKTKPREEQYSSTYRVVSVLTVLHQDWLNGKEYKCKVSNKALPAPIEKTISKAKGQPREPQVYTKPPSREEMTKNQVSLSCLVKGFYPSDIAVEWESNGQPENNYKTTVPVLDSDGSFRLASYLTVDKSRWQQGNVFSCSVMHEALHNHYTQKSLSLSPGSTGSEVQLQQSGPELVKPGASVKISCKTSGYTFTEYTMHWVKQSHGKSLEWIGGISPNIGGTSYNQKFKGKATLTVDKSSSTAYMELRSLTSEDSAVYYCARRGGSFDYWGQGTTLTVSSRTVAAPSVFIFPPSDEQLKSGTASVVCLLNNFYPREAKVQWKVDNALQSGNSQESVTEQDSKDSTYSLSSTLTLSKADYEKHKVYACEVTHQGLSSPVTKSFNRGEC

SEQ ID NO: 15 - protein, 214 aa, Artificial
  Chimeric homo sapiens mus musculus
DIVMTQSPATLSVTPGDRVSLSCRASQSISDYLHWYQQKSHESPRLLIKYASQSISGIPSRFSGSGSGSDFTLSINSVEPEDVGVYYCQNGHSFPLTFGAGTKLELKASTKGPSVFPLAPSSKSTSGGTAALGCLVKDYFPEPVTVSWNSGALTSGVHTFPAVLQSSGLYSLSSVVTVPSSSLGTQTYICNVNHKPSNTKVDKRVEPKSCDKTH

SEQ ID NO: 16 - protein, 218 aa, Artificial; identical to SEQ ID NO: 13
  Chimeric homo sapiens mus musculus

SEQ ID NO: 17 - protein, 801 aa, Artificial
  Chimeric homo sapiens mus musculus
QVQLQQSGAELVRPGSSVKISCKASGYAFSSYWMNWVKQRPGQGLEWIGQIWPGDGDTNYNGKFKGKATLTADESSSTAYMQLSSLASEDSAVYFCARRETTTVGRYYYAMDYWGQGTTVTVSSASTKGPSVFPLAPSSKSTSGGTAALGCLVKDYFPEPVTVSWNSGALTSGVHTFPAVLQSSGLYSLSSVVTVPSSSLGTQTYICNVNHKPSNTKVDKRVEPKSCDKTHTCPPCPAPELLGGPSVFLFPPKPKDTLMISRTPEVTCVVVDVSHEDPEVKFNWYVDGVEVHNAKTKPREEQYSSTYRVVSVLTVLHQDWLNGKEYKCKVSNKALPAPIEKTISKAKGQPREPQVYTLPPSREEMTKNQVSLTCLVKGFYPSDIAVEWESNGQPENNYKTTPPVLDSDGSFFLYSKLTVDKSRWQQGNVFSCSVMHEALHNHYTQKSLSLSPGGGGGSGGGGSGGGGSGQPREPQVYTLPPSREEMTKNQVSLTCLVKGFYPSDIAVEWESNGQPENNYKTTPPVLDSDGSFFLYSKLTVDKSRWQQGNVFSCSVMHEALHNHYTQKSLSLSPGSTGSEVQLQQSGPELVKPGASVKISCKTSGYTFTEYTMHWVKQSHGKSLEWIGGISPNIGGTSYNQKFKGKATLTVDKSSSTAYMELRSLTSEDSAVYYCARRGGSFDYWGQGTTLTVSSRTVAAPSVFIFPPSDEQLKSGTASVVCLLNNFYPREAKVQWKVDNALQSGNSQESVTEQDSKDSTYSLSSTLTLSKADYEKHKVYACEVTHQGLSSPVTKSFNRGEC

SEQ ID NO: 18 - protein, 214 aa, Artificial; identical to SEQ ID NO: 15
  Chimeric homo sapiens mus musculus

SEQ ID NO: 19 - protein, 218 aa, Artificial; identical to SEQ ID NO: 13
  Chimeric homo sapiens mus musculus

SEQ ID NO: 20 - protein, 801 aa, Artificial
  Chimeric homo sapiens mus musculus
QVQLQQSGAELVRPGSSVKISCKASGYAFSSYWMNWVKQRPGQGLEWIGQIWPGDGDTNYNGKFKGKATLTADESSSTAYMQLSSLASEDSAVYFCARRETTTVGRYYYAMDYWGQGTTVTVSSASTKGPSVFPLAPSSKSTSGGTAALGCLVKDYFPEPVTVSWNSGALTSGVHTFPAVLQSSGLYSLSSVVTVPSSSLGTQTYICNVNHKPSNTKVDKRVEPKSCDKTHTSPPSPAPELLGGPSVFLFPPKPKDTLMISRTPEVTCVVVDVSHEDPEVKFNWYVDGVEVHNAKTKPREEQYSSTYRVVSVLTVLHQDWLNGKEYKCKVSNKALPAPIEKTISKAKGQPREPQVYTLPPSREEMTKNQVSLTCLVKGFYPSDIAVEWESNGQPENNYKTTPPVLDSDGSFFLYSKLTVDKSRWQQGNVFSCSVMHEALHNHYTQKSLSLSPGGGGGSGGGGSGGGGSGQPREPQVYTLPPSREEMTKNQVSLTCLVKGFYPSDIAVEWESNGQPENNYKTTPPVLDSDGSFFLYSKLTVDKSRWQQGNVFSCSVMHEALHNHYTQKSLSLSPGSTGSEVQLQQSGPELVKPGASVKISCKTSGYTFTEYTMHWVKQSHGKSLEWIGGISPNIGGTSYNQKFKGKATLTVDKSSSTAYMELRSLTSEDSAVYYCARRGGSFDYWGQGTTLTVSSRTVAAPSVFIFPPSDEQLKSGTASVVCLLNNFYPREAKVQWKVDNALQSGNSQESVTEQDSKDSTYSLSSTLTLSKADYEKHKVYACEVTHQGLSSPVTKSFNRGEC

SEQ ID NO: 21 - protein, 214 aa, Artificial; identical to SEQ ID NO: 15
  Chimeric homo sapiens mus musculus

SEQ ID NO: 22 - protein, 218 aa, Artificial; identical to SEQ ID NO: 13
  Chimeric homo sapiens mus musculus

SEQ ID NO: 23 - protein, 796 aa, Artificial
  Chimeric homo sapiens mus musculus
QVQLQQSGAELVRPGSSVKISCKASGYAFSSYWMNWVKQRPGQGLEWIGQIWPGDGDTNYNGKFKGKATLTADESSSTAYMQLSSLASEDSAVYFCARRETTTVGRYYYAMDYWGQGTTVTVSSASTKGPSVFPLAPSSKSTSGGTAALGCLVKDYFPEPVTVSWNSGALTSGVHTFPAVLQSSGLYSLSSVVTVPSSSLGTQTYICNVNHKPSNTKVDKRVEPKSCGGGSSAPELLGGPSVFLFPPKPKDTLMISRTPEVTCVVVDVSHEDPEVKFNWYVDGVEVHNAKTKPREEQYSSTYRVVSVLTVLHQDWLNGKEYKCKVSNKALPAPIEKTISKAKGQPREPQVYTLPPSREEMTKNQVSLTCLVKGFYPSDIAVEWESNGQPENNYKTTPPVLDSDGSFFLYSKLTVDKSRWQQGNVFSCSVMHEALHNHYTQKSLSLSPGGGGGSGGGGSGGGGSGQPREPQVYTLPPSREEMTKNQVSLTCLVKGFYPSDIAVEWESNGQPENNYKTTPPVLDSDGSFFLYSKLTVDKSRWQQGNVFSCSVMHEALHNHYTQKSLSLSPGSTGSEVQLQQSGPELVKPGASVKISCKTSGYTFTEYTMHWVKQSHGKSLEWIGGISPNIGGTSYNQKFKGKATLTVDKSSSTAYMELRSLTSEDSAVYYCARRGGSFDYWGQGTTLTVSSRTVAAPSVFIFPPSDEQLKSGTASVVCLLNNFYPREAKVQWKVDNALQSGNSQESVTEQDSKDSTYSLSSTLTLSKADYEKHKVYACEVTHQGLSSPVTKSFNRGEC

SEQ ID NO: 24 - protein, 214 aa, Artificial; identical to SEQ ID NO: 15
  Chimeric homo sapiens mus musculus

SEQ ID NO: 25 - protein, 218 aa, Artificial; identical to SEQ ID NO: 13
  Chimeric homo sapiens mus musculus

SEQ ID NO: 26 - protein, 819 aa, Artificial
  Chimeric homo sapiens mus musculus
QVQLQQSGAELVRPGSSVKISCKASGYAFSSYWMNWVKQRPGQGLEWIGQIWPGDGDTNYNGKFKGKATLTADESSSTAYMQLSSLASEDSAVYFCARRETTTVGRYYYAMDYWGQGTTVTVSSASTKGPSVFPLAPSSKSTSGGTAALGCLVKDYFPEPVTVSWNSGALTSGVHTFPAVLQSSGLYSLSSVVTVPSSSLGTQTYICNVNHKPSNTKVDKRVEPKSCDKTHTCPPCPAPELLGGPSVFLFPPKPKDTLMISRTPEVTCVVVDVSHEDPEVKFNWYVDGVEVHNAKTKPREEQYSSTYRVVSVLTVLHQDWLNGKEYKCKVSNKALPAPIEKTISKAKGQPREPQVYTLPPSREEMTKNQVSLTCLVKGFYPSDIAVEWESNGQPENNYKTTPPVLDSDGSFFLYSKLTVDKSRWQQGNVFSCSVMHEALHNHYTQKSLSLSPGGGGGSGGGGSGGGGSGQPREPQVYTLPPSREEMTKNQVSLTCLVKGFYPSDIAVEWESNGQPENNYKTTPPVLDSDGSFFLYSKLTVDKSRWQQGNVFSCSVMHEALHNHYTQKSLSLSPGSTGSEVQLQQSGPELVKPGASVKISCKTSGYTFTEYTMHWVKQSHGKSLEWIGGISPNIGGTSYNQKFKGKATLTVDKSSSTAYMELRSLTSEDSAVYYCARRGGSFDYWGQGTTLTVSSVEGGSGGSGGSGGSGGVDDIVMTQSPATLSVTPGDRVSLSCRASQSISDYLHWYQQKSHESPRLLIKYASQSISGIPSRFSGSGSGSDFTLSINSVEPEDVGVYYCQNGHSFPLTFGAGTKLELK

SEQ ID NO: 27 - protein, 218 aa, Artificial; identical to SEQ ID NO: 13
  Chimeric homo sapiens mus musculus

SEQ ID NO: 28 - protein, 819 aa, Artificial
  Chimeric homo sapiens mus musculus
QVQLQQSGAELVRPGSSVKISCKASGYAFSSYWMNWVKQRPGQGLEWIGQIWPGDGDTNYNGKFKGKATLTADESSSTAYMQLSSLASEDSAVYFCARRETTTVGRYYYAMDYWGQGTTVTVSSASTKGPSVFPLAPSSKSTSGGTAALGCLVKDYFPEPVTVSWNSGALTSGVHTFPAVLQSSGLYSLSSVVTVPSSSLGTQTYICNVNHKPSNTKVDKRVEPKSCDKTHTSPPSPAPELLGGPSVFLFPPKPKDTLMISRTPEVTCVVVDVSHEDPEVKFNWYVDGVEVHNAKTKPREEQYSSTYRVVSVLTVLHQDWLNGKEYKCKVSNKALPAPIEKTISKAKGQPREPQVYTLPPSREEMTKNQVSLTCLVKGFYPSDIAVEWESNGQPENNYKTTPPVLDSDGSFFLYSKLTVDKSRWQQGNVFSCSVMHEALHNHYTQKSLSLSPGGGGGSGGGGSGGGGSGQPREPQVYTLPPSREEMTKNQVSLTCLVKGFYPSDIAVEWESNGQPENNYKTTPPVLDSDGSFFLYSKLTVDKSRWQQGNVFSCSVMHEALHNHYTQKSLSLSPGSTGSEVQLQQSGPELVKPGASVKISCKTSGYTFTEYTMHWVKQSHGKSLEWIGGISPNIGGTSYNQKFKGKATLTVDKSSSTAYMELRSLTSEDSAVYYCARRGGSFDYWGQGTTLTVSSVEGGSGGSGGSGGSGGVDDIVMTQSPATLSVTPGDRVSLSCRASQSISDYLHWYQQKSHESPRLLIKYASQSISGIPSRFSGSGSGSDFTLSINSVEPEDVGVYYCQNGHSFPLTFGAGTKLELK

SEQ ID NO: 29 - protein, 218 aa, Artificial; identical to SEQ ID NO: 13
  Chimeric homo sapiens mus musculus

SEQ ID NO: 30 - protein, 815 aa, Artificial
  Chimeric homo sapiens mus musculus
QVQLQQSGAELVRPGSSVKISCKASGYAFSSYWMNWVKQRPGQGLEWIGQIWPGDGDTNYNGKFKGKATLTADESSSTAYMQLSSLASEDSAVYFCARRETTTVGRYYYAMDYWGQGTTVTVSSASTKGPSVFPLAPSSKSTSGGTAALGCLVKDYFPEPVTVSWNSGALTSGVHTFPAVLQSSGLYSLSSVVTVPSSSLGTQTYICNVNHKPSNTKVDKRVEPKSCGGGSSPAPELLGGPSVFLFPPKPKDTLMISRTPEVTCVVVDVSHEDPEVKFNWYVDGVEVHNAKTKPREEQYSSTYRVVSVLTVLHQDWLNGKEYKCKVSNKALPAPIEKTISKAKGQPREPQVYTLPPSREEMTKNQVSLTCLVKGFYPSDIAVEWESNGQPENNYKTTPPVLDSDGSFFLYSKLTVDKSRWQQGNVFSCSVMHEALHNHYTQKSLSLSPGGGGGSGGGGSGGGGSGQPREPQVYTLPPSREEMTKNQVSLTCLVKGFYPSDIAVEWESNGQPENNYKTTPPVLDSDGSFFLYSKLTVDKSRWQQGNVFSCSVMHEALHNHYTQKSLSLSPGSTGSEVQLQQSGPELVKPGASVKISCKTSGYTFTEYTMHWVKQSHGKSLEWIGGISPNIGGTSYNQKFKGKATLTVDKSSSTAYMELRSLTSEDSAVYYCARRGGSFDYWGQGTTLTVSSVEGGSGGSGGSGGSGGVDDIVMTQSPATLSVTPGDRVSLSCRASQSISDYLHWYQQKSHESPRLLIKYASQSISGIPSRFSGSGSGSDFTLSINSVEPEDVGVYYCQNGHSFPLTFGAGTKLELK

SEQ ID NO: 31 - protein, 819 aa, Artificial
  Chimeric homo sapiens mus musculus
DIQLTQSPASLAVSLGQRATISCKASQSVDYDGDSYLNWYQQIPGQPPKLLIYDASNLVSGIPPRFSGSGSGTDFTLNIHPVEKVDAATYHCQQSTEDPWTFGGGTKLEIKGGGGSGGGGSGGGGSQVQLQQSGAELVRPGSSVKISCKASGYAFSSYWMNWVKQRPGQGLEWIGQIWPGDGDTNYNGKFKGKATLTADESSSTAYMQLSSLASEDSAVYFCARRETTTVGRYYYAMDYWGQGTTVTVSSGGGSSAPELLGGPSVFLFPPKPKDTLMISRTPEVTCVVVDVSHEDPEVKFNWYVDGVEVHNAKTKPREEQYSSTYRVVSVLTVLHQDWLNGKEYKCKVSNKALPAPIEKTISKAKGQPREPQVYTLPPSREEMTKNQVSLTCLVKGFYPSDIAVEWESNGQPENNYKTTPPVLDSDGSFFLYSKLTVDKSRWQQGNVFSCSVMHEALHNHYTQKSLSLSPGGGGGSGGGGSGGGGSGQPREPQVYTLPPSREEMTKNQVSLTCLVKGFYPSDIAVEWESNGQPENNYKTTPPVLDSDGSFFLYSKLTVDKSRWQQGNVFSCSVMHEALHNHYTQKSLSLSPGSTGSEVQLQQSGPELVKPGASVKISCKTSGYTFTEYTMHWVKQSHGKSLEWIGGISPNIGGTSYNQKFKGKATLTVDKSSSTAYMELRSLTSEDSAVYYCARRGGSFDYWGQGTTLTVSSRTVAAPSVFIFPPSDEQLKSGTASVVCLLNNFYPREAKVQWKVDNALQSGNSQESVTEQDSKDSTYSLSSTLTLSKADYEKHKVYACEVTHQGLSSPVTKSFNRGEC

SEQ ID NO: 32 - protein, 214 aa, Artificial; identical to SEQ ID NO: 15
  Chimeric homo sapiens mus musculus

SEQ ID NO: 33 - protein, 819 aa, Artificial
  Chimeric homo sapiens mus musculus
DIQLTQSPASLAVSLGQRATISCKASQSVDYDGDSYLNWYQQIPGQPPKLLIYDASNLVSGIPPRFSGSGSGTDFTLNIHPVEKVDAATYHCQQSTEDPWTFGGGTKLEIKGGGGSGGGGSGGGGSQVQLQQSGAELVRPGSSVKISCKASGYAFSSYWMNWVKQRPGQGLEWIGQIWPGDGDTNYNGKFKGKATLTADESSSTAYMQLSSLASEDSAVYFCARRETTTVGRYYYAMDYWGQGTTVTVSSGGGSSAPELLGGPSVFLFPPKPKDTLMISRTPEVTCVVVDVSHEDPEVKFNWYVDGVEVHNAKTKPREEQYSSTYRVVSVLTVLHQDWLNGKEYKCKVSNKALPAPIEKTISKAKGQPREPQVYTLPPSREEMTKNQVSLTCLVKGFYPSDIAVEWESNGQPENNYKTTPPVLDSDGSFFLYSKLTVDKSRWQQGNVFSCSVMHEALHNHYTQKSLSLSPGGGGGSGGGGSGGGGSGQPREPQVYTLPPSREEMTKNQVSLTCLVKGFYPSDIAVEWESNGQPENNYKTTPPVLDSDGSFFLYSKLTVDKSRWQQGNVFSCSVMHEALHNHYTQKSLSLSPGSTGSEVQLQQSGPELVKPGASVKISCKTSGYTFTEYTMHWVKQSHGKSLEWIGGISPNIGGTSYNQKFKGKATLTVDKSSSTAYMELRSLTSEDSAVYYCARRGGSFDYWGQGTTLTVSSASTKGPSVFPLAPSSKSTSGGTAALGCLVKDYFPEPVTVSWNSGALTSGVHTFPAVLQSSGLYSLSSVVTVPSSSLGTQTYICNVNHKPSNTKVDKRVEPKSCDKTH

SEQ ID NO: 34 - protein, 214 aa, Artificial; identical to SEQ ID NO: 12
  Chimeric homo sapiens mus musculus

SEQ ID NO: 35 - protein, 218 aa, Artificial; identical to SEQ ID NO: 13
  Chimeric homo sapiens mus musculus

SEQ ID NO: 36 - protein, 792 aa, Artificial
  Chimeric homo sapiens mus musculus
QVQLQQSGAELVRPGSSVKISCKASGYAFSSYWMNWVKQRPGQGLEWIGQIWPGDGDTNYNGKFKGKATLTADESSSTAYMQLSSLASEDSAVYFCARRETTTVGRYYYAMDYWGQGTTVTVSSASTKGPSVFPLAPSSKSTSGGTAALGCLVKDYFPEPVTVSWNSGALTSGVHTFPAVLQSSGLYSLSSVVTVPSSSLGTQTYICNVNHKPSNTKVDKRVEPKSCDKTHTSPPSPAPELLGGPSVFLFPPKPKDTLMISRTPEVTCVVVDVSHEDPEVKFNWYVDGVEVHNAKTKPREEQYSSTYRVVSVLTVLHQDWLNGKEYKCKVSNKALPAPIEKTISKAKGQPREPQVYTLPPSREEMTKNQVSLTCLVKGFYPSDIAVEWESNGQPENNYKTTPPVLDSDGSFFLYSKLTVDKSRWQQGNVFSCSVMHEALHNHYTQKSLSLSPGGGGGSGGGGSGGGGSGQPREPQVYTLPPSREEMTKNQVSLTCLVKGFYPSDIAVEWESNGQPENNYKTTPPVLDSDGSFFLYSKLTVDKSRWQQGNVFSCSVMHEALHNHYTQKSLSLSPGSTGSDIVMTQSPATLSVTPGDRVSLSCRASQSISDYLHWYQQKSHESPRLLIKYASQSISGIPSRFSGSGSGSDFTLSINSVEPEDVGVYYCQNGHSFPLTFGAGTKLELKASTKGPSVFPLAPSSKSTSGGTAALGCLVKDYFPEPVTVSWNSGALTSGVHTFPAVLQSSGLYSLSSVVTVPSSSLGTQTYICNVNHKPSNTKVDKRVEPKSCDKTH

SEQ ID NO: 37 - protein, 223 aa, Artificial
  Chimeric homo sapiens mus musculus
EVQLQQSGPELVKPGASVKISCKTSGYTFTEYTMHWVKQSHGKSLEWIGGISPNIGGTSYNQKFKGKATLTVDKSSSTAYMELRSLTSEDSAVYYCARRGGSFDYWGQGTTLTVSSRTVAAPSVFIFPPSDEQLKSGTASVVCLLNNFYPREAKVQWKVDNALQSGNSQESVTEQDSKDSTYSLSSTLTLSKADYEKHKVYACEVTHQGLSSPVTKSFNRGEC

SEQ ID NO: 38 - protein, 445 aa, Artificial
  Chimeric homo sapiens mus musculus
DIQLTQSPASLAVSLGQRATISCKASQSVDYDGDSYLNWYQQIPGQPPKLLIYDASNLVSGIPPRFSGSGSGTDFTLNIHPVEKVDAATYHCQQSTEDPWTFGGGTKLEIKRTVAAPSVFIFPPSDEQLKSGTASVVCLLNNFYPREAKVQWKVDNALQSGNSQESVTEQDSKDSTYSLSSTLTLSKADYEKHKVYACEVTHQGLSSPVTKSFNRGECDKTHTCPPCPAPELLGGPSVFLFPPKPKDTLMISRTPEVTCVVVDVSHEDPEVKFNWYVDGVEVHNAKTKPREEQYNSTYRVVSVLTVLHQDWLNGKEYKCKVSNKALPAPIEKTISKAKGQPREPQVYTLPPSREEMTKNQVSLTCLVKGFYPSDIAVEWESNGQPENNYKTTPPVLDSDGSFFLYSKLTVDKSRWQQGNVFSCSVMHEALHNHYTQKSLSLSPGK

SEQ ID NO: 39 - protein, 680 aa, Artificial
  Chimeric homo sapiens mus musculus
QVQLQQSGAELVRPGSSVKISCKASGYAFSSYWMNWVKQRPGQGLEWIGQIWPGDGDTNYNGKFKGKATLTADESSSTAYMQLSSLASEDSAVYFCARRETTTVGRYYYAMDYWGQGTTVTVSSASTKGPSVFPLAPSSKSTSGGTAALGCLVKDYFPEPVTVSWNSGALTSGVHTFPAVLQSSGLYSLSSVVTVPSSSLGTQTYICNVNHKPSNTKVDKRVEPKSCDKTHTCPPCPAPELLGGPSVFLFPPKPKDTLMISRTPEVTCVVVDVSHEDPEVKFNWYVDGVEVHNAKTKPREEQYNSTYRVVSVLTVLHQDWLNGKEYKCKVSNKALPAPIEKTISKAKGQPREPQVYTLPPSREEMTKNQVSLTCLVKGFYPSDIAVEWESNGQPENNYKTTPPVLDSDGSFFLYSKLTVDKSRWQQGNVFSCSVMHEALHNHYTQKSLSLSPGSTGSEVQLQQSGPELVKPGASVKISCKTSGYTFTEYTMHWVKQSHGKSLEWIGGISPNIGGTSYNQKFKGKATLTVDKSSSTAYMELRSLTSEDSAVYYCARRGGSFDYWGQGTTLTVSSRTVAAPSVFIFPPSDEQLKSGTASVVCLLNNFYPREAKVQWKVDNALQSGNSQESVTEQDSKDSTYSLSSTLTLSKADYEKHKVYACEVTHQGLSSPVTKSFNRGEC

SEQ ID NO: 40 - protein, 214 aa, Artificial; identical to SEQ ID NO: 15
  Chimeric homo sapiens mus musculus

SEQ ID NO: 41 - protein, 445 aa, Artificial
  Chimeric homo sapiens mus musculus
DIQLTQSPASLAVSLGQRATISCKASQSVDYDGDSYLNWYQQIPGQPPKLLIYDASNLVSGIPPRFSGSGSGTDFTLNIHPVEKVDAATYHCQQSTEDPWTFGGGTKLEIKRTVAAPSVFIFPPSDEQLKSGTASVVCLLNNFYPREAKVQWKVDNALQSGNSQESVTEQDSKDSTYSLSSTLTLSKADYEKHKVYACEVTHQGLSSPVTKSFNRGECDKTHTCPPCPAPELLGGPSVFLFPPKPKDTLMISRTPEVTCVVVDVSHEDPEVKFNWYVDGVEVHNAKTKPREEQYSSTYRVVSVLTVLHQDWLNGKEYKCKVSNKALPAPIEKTISKAKGQPREPQVYTLPPSREEMTKNQVSLTCLVKGFYPSDIAVEWESNGQPENNYKTTPPVLDSDGSFFLYSKLTVDKSRWQQGNVFSCSVMHEALHNHYTQKSLSLSPGK

SEQ ID NO: 42 - protein, 680 aa, Artificial
  Chimeric homo sapiens mus musculus
QVQLQQSGAELVRPGSSVKISCKASGYAFSSYWMNWVKQRPGQGLEWIGQIWPGDGDTNYNGKFKGKATLTADESSSTAYMQLSSLASEDSAVYFCARRETTTVGRYYYAMDYWGQGTTVTVSSASTKGPSVFPLAPSSKSTSGGTAALGCLVKDYFPEPVTVSWNSGALTSGVHTFPAVLQSSGLYSLSSVVTVPSSSLGTQTYICNVNHKPSNTKVDKRVEPKSCDKTHTCPPCPAPELLGGPSVFLFPPKPKDTLMISRTPEVTCVVVDVSHEDPEVKFNWYVDGVEVHNAKTKPREEQYSSTYRVVSVLTVLHQDWLNGKEYKCKVSNKALPAPIEKTISKAKGQPREPQVYTLPPSREEMTKNQVSLTCLVKGFYPSDIAVEWESNGQPENNYKTTPPVLDSDGSFFLYSKLTVDKSRWQQGNVFSCSVMHEALHNHYTQKSLSLSPGSTGSEVQLQQSGPELVKPGASVKISCKTSGYTFTEYTMHWVKQSHGKSLEWIGGISPNIGGTSYNQKFKGKATLTVDKSSSTAYMELRSLTSEDSAVYYCARRGGSFDYWGQGTTLTVSSRTVAAPSVFIFPPSDEQLKSGTASVVCLLNNFYPREAKVQWKVDNALQSGNSQESVTEQDSKDSTYSLSSTLTLSKADYEKHKVYACEVTHQGLSSPVTKSFNRGEC

SEQ ID NO: 43 - protein, 214 aa, Artificial; identical to SEQ ID NO: 15
  Chimeric homo sapiens mus musculus

SEQ ID NO: 44 - protein, 445 aa, Artificial
  Chimeric homo sapiens mus musculus
DIQLTQSPASLAVSLGQRATISCKASQSVDYDGDSYLNWYQQIPGQPPKLLIYDASNLVSGIPPRFSGSGSGTDFTLNIHPVEKVDAATYHCQQSTEDPWTFGGGTKLEIKRTVAAPSVFIFPPSDEQLKSGTASVVCLLNNFYPREAKVQWKVDNALQSGNSQESVTEQDSKDSTYSLSSTLTLSKADYEKHKVYACEVTHQGLSSPVTKSFNRGESDKTHTCPPCPAPELLGGPSVFLFPPKPKDTLMISRTPEVTCVVVDVSHEDPEVKFNWYVDGVEVHNAKTKPREEQYSSTYRVVSVLTVLHQDWLNGKEYKCKVSNKALPAPIEKTISKAKGQPREPQVYTLPPSREEMTKNQVSLTCLVKGFYPSDIAVEWESNGQPENNYKTTPPVLDSDGSFFLYSKLTVDKSRWQQGNVFSCSVMHEALHNHYTQKSLSLSPGK

SEQ ID NO: 45 - protein, 680 aa, Artificial
  Chimeric homo sapiens mus musculus
QVQLQQSGAELVRPGSSVKISCKASGYAFSSYWMNWVKQRPGQGLEWIGQIWPGDGDTNYNGKFKGKATLTADESSSTAYMQLSSLASEDSAVYFCARRETTTVGRYYYAMDYWGQGTTVTVSSASTKGPSVFPLAPSSKSTSGGTAALGCLVKDYFPEPVTVSWNSGALTSGVHTFPAVLQSSGLYSLSSVVTVPSSSLGTQTYICNVNHKPSNTKVDKRVEPKSSDKTHTCPPCPAPELLGGPSVFLFPPKPKDTLMISRTPEVTCVVVDVSHEDPEVKFNWYVDGVEVHNAKTKPREEQYSSTYRVVSVLTVLHQDWLNGKEYKCKVSNKALPAPIEKTISKAKGQPREPQVYTLPPSREEMTKNQVSLTCLVKGFYPSDIAVEWESNGQPENNYKTTPPVLDSDGSFFLYSKLTVDKSRWQQGNVFSCSVMHEALHNHYTQKSLSLSPGSTGSEVQLQQSGPELVKPGASVKISCKTSGYTFTEYTMHWVKQSHGKSLEWIGGISPNIGGTSYNQKFKGKATLTVDKSSSTAYMELRSLTSEDSAVYYCARRGGSFDYWGQGTTLTVSSRTVAAPSVFIFPPSDEQLKSGTASVVCLLNNFYPREAKVQWKVDNALQSGNSQESVTEQDSKDSTYSLSSTLTLSKADYEKHKVYACEVTHQGLSSPVTKSFNRGEC

SEQ ID NO: 46 - protein, 214 aa, Artificial; identical to SEQ ID NO: 15
  Chimeric homo sapiens mus musculus

SEQ ID NO: 47 - protein, 445 aa, Artificial; identical to SEQ ID NO: 38
  Chimeric homo sapiens mus musculus

SEQ ID NO: 48 - protein, 698 aa, Artificial
  Chimeric homo sapiens mus musculus
QVQLQQSGAELVRPGSSVKISCKASGYAFSSYWMNWVKQRPGQGLEWIGQIWPGDGDTNYNGKFKGKATLTADESSSTAYMQLSSLASEDSAVYFCARRETTTVGRYYYAMDYWGQGTTVTVSSASTKGPSVFPLAPSSKSTSGGTAALGCLVKDYFPEPVTVSWNSGALTSGVHTFPAVLQSSGLYSLSSVVTVPSSSLGTQTYICNVNHKPSNTKVDKRVEPKSCDKTHTCPPCPAPELLGGPSVFLFPPKPKDTLMISRTPEVTCVVVDVSHEDPEVKFNWYVDGVEVHNAKTKPREEQYNSTYRVVSVLTVLHQDWLNGKEYKCKVSNKALPAPIEKTISKAKGQPREPQVYTLPPSREEMTKNQVSLTCLVKGFYPSDIAVEWESNGQPENNYKTTPPVLDSDGSFFLYSKLTVDKSRWQQGNVFSCSVMHEALHNHYTQKSLSLSPGSTGSEVQLQQSGPELVKPGASVKISCKTSGYTFTEYTMHWVKQSHGKSLEWIGGISPNIGGTSYNQKFKGKATLTVDKSSSTAYMELRSLTSEDSAVYYCARRGGSFDYWGQGTTLTVSSVEGGSGGSGGSGGSGGVDDIVMTQSPATLSVTPGDRVSLSCRASQSISDYLHWYQQKSHESPRLLIKYASQSISGIPSRFSGSGSGSDFTLSINSVEPEDVGVYYCQNGHSFPLTFGAGTKLELK

SEQ ID NO: 49 - protein, 444 aa, Artificial
  Chimeric homo sapiens mus musculus
IQLTQSPASLAVSLGQRATISCKASQSVDYDGDSYLNWYQQIPGQPPKLLIYDASNLVSGIPPRFSGSGSGTDFTLNIHPVEKVDAATYHCQQSTEDPWTFGGGTKLEIKRTVAAPSVFIFPPSDEQLKSGTASVVCLLNNFYPREAKVQWKVDNALQSGNSQESVTEQDSKDSTYSLSSTLTLSKADYEKHKVYACEVTHQGLSSPVTKSFNRGECDKTHTCPPCPAPELLGGPSVFLFPPKPKDTLMISRTPEVTCVVVDVSHEDPEVKFNWYVDGVEVHNAKTKPREEQYSSTYRVVSVLTVLHQDWLNGKEYKCKVSNKALPAPIEKTISKAKGQPREPQVYTLPPSREEMTKNQVSLTCLVKGFYPSDIAVEWESNGQPENNYKTTPPVLDSDGSFFLYSKLTVDKSRWQQGNVFSCSVMHEALHNHYTQKSLSLSPGK

SEQ ID NO: 50 - protein, 698 aa, Artificial
  Chimeric homo sapiens mus musculus
QVQLQQSGAELVRPGSSVKISCKASGYAFSSYWMNWVKQRPGQGLEWIGQIWPGDGDTNYNGKFKGKATLTADESSSTAYMQLSSLASEDSAVYFCARRETTTVGRYYYAMDYWGQGTTVTVSSASTKGPSVFPLAPSSKSTSGGTAALGCLVKDYFPEPVTVSWNSGALTSGVHTFPAVLQSSGLYSLSSVVTVPSSSLGTQTYICNVNHKPSNTKVDKRVEPKSCDKTHTCPPCPAPELLGGPSVFLFPPKPKDTLMISRTPEVTCVVVDVSHEDPEVKFNWYVDGVEVHNAKTKPREEQYSSTYRVVSVLTVLHQDWLNGKEYKCKVSNKALPAPIEKTISKAKGQPREPQVYTLPPSREEMTKNQVSLTCLVKGFYPSDIAVEWESNGQPENNYKTTPPVLDSDGSFFLYSKLTVDKSRWQQGNVFSCSVMHEALHNHYTQKSLSLSPGSTGSEVQLQQSGPELVKPGASVKISCKTSGYTFTEYTMHWVKQSHGKSLEWIGGISPNIGGTSYNQKFKGKATLTVDKSSSTAYMELRSLTSEDSAVYYCARRGGSFDYWGQGTTLTVSSVEGGSGGSGGSGGSGGVDDIVMTQSPATLSVTPGDRVSLSCRASQSISDYLHWYQQKSHESPRLLIKYASQSISGIPSRFSGSGSGSDFTLSINSVEPEDVGVYYCQNGHSFPLTFGAGTKLELK

SEQ ID NO: 51 - protein, 454 aa, Artificial
  Chimeric homo sapiens mus musculus
QVQLQQSGAELVRPGSSVKISCKASGYAFSSYWMNWVKQRPGQGLEWIGQIWPGDGDTNYNGKFKGKATLTADESSSTAYMQLSSLASEDSAVYFCARRETTTVGRYYYAMDYWGQGTTVTVSSASTKGPSVFPLAPSSKSTSGGTAALGCLVKDYFPEPVTVSWNSGALTSGVHTFPAVLQSSGLYSLSSVVTVPSSSLGTQTYICNVNHKPSNTKVDKRVEPKSCDKTHTCPPCPAPELLGGPSVFLFPPKPKDTLMISRTPEVTCVVVDVSHEDPEVKFNWYVDGVEVHNAKTKPREEQYSSTYRVVSVLTVLHQDWLNGKEYKCKVSNKALPAPIEKTISKAKGQPREPQVYTLPPSREEMTKNQVSLTCLVKGFYPSDIAVEWESNGQPENNYKTTPPVLDSDGSFFLYSKLTVDKSRWQQGNVFSCSVMHEALHNHYTQKSLSLSPGK

SEQ ID NO: 52 - protein, 670 aa, Artificial
  Chimeric homo sapiens mus musculus
DIQLTQSPASLAVSLGQRATISCKASQSVDYDGDSYLNWYQQIPGQPPKLLIYDASNLVSGIPPRFSGSGSGTDFTLNIHPVEKVDAATYHCQQSTEDPWTFGGGTKLEIKRTVAAPSVFIFPPSDEQLKSGTASVVCLLNNFYPREAKVQWKVDNALQSGNSQESVTEQDSKDSTYSLSSTLTLSKADYEKHKVYACEVTHQGLSSPVTKSFNRGECDKTHTCPPCPAPELLGGPSVFLFPPKPKDTLMISRTPEVTCVVVDVSHEDPEVKFNWYVDGVEVHNAKTKPREEQSSTYRVVSVLTVLHQDWLNGKEYKCKVSNKALPAPIEKTISKAKGQPREPQVYTLPPSREEMTKNQVSLTCLVKGFYPSDIAVEWESNGQPENNYKTTPPVLDSDGSFFLYSKLTVDKSRWQQGNVFSCSVMHEALHNHYTQKSLSLSPGSTGSEVQLQQSGPELVKPGASVKISCKTSGYTFTEYTMHWVKQSHGKSLEWIGGISPNIGGTSYNQKFKGKATLTVDKSSSTAYMELRSLTSEDSAVYYCARRGGSFDYWGQGTTLTVSSRTVAAPSVFIFPPSDEQLKSGTASVVCLLNNFYPREAKVQWKVDNALQSGNSQESVTEQDSKDSTYSLSSTLTLSKADYEKHKVYACEVTHQGLSSPVTKSFNRGEC

SEQ ID NO: 53 - protein, 214 aa, Artificial; identical to SEQ ID NO: 15
  Chimeric homo sapiens mus musculus

SEQ ID NO: 54 - protein, 445 aa, Artificial; identical to SEQ ID NO: 41
  Chimeric homo sapiens mus musculus

SEQ ID NO: 55 - protein, 671 aa, Artificial
  Chimeric homo sapiens mus musculus
QVQLQQSGAELVRPGSSVKISCKASGYAFSSYWMNWVKQRPGQGLEWIGQIWPGDGDTNYNGKFKGKATLTADESSSTAYMQLSSLASEDSAVYFCARRETTTVGRYYYAMDYWGQGTTVTVSSASTKGPSVFPLAPSSKSTSGGTAALGCLVKDYFPEPVTVSWNSGALTSGVHTFPAVLQSSGLYSLSSVVTVPSSSLGTQTYICNVNHKPSNTKVDKRVEPKSCDKTHTCPPCPAPELLGGPSVFLFPPKPKDTLMISRTPEVTCVVVDVSHEDPEVKFNWYVDGVEVHNAKTKPREEQYSSTYRVVSVLTVLHQDWLNGKEYKCKVSNKALPAPIEKTISKAKGQPREPQVYTLPPSREEMTKNQVSLTCLVKGFYPSDIAVEWESNGQPENNYKTTPPVLDSDGSFFLYSKLTVDKSRWQQGNVFSCSVMHEALHNHYTQKSLSLSPGSTGSDIVMTQSPATLSVTPGDRVSLSCRASQSISDYLHWYQQKSHESPRLLIKYASQSISGIPSRFSGSGSGSDFTLSINSVEPEDVGVYYCQNGHSFPLTFGAGTKLELKASTKGPSVFPLAPSSKSTSGGTAALGCLVKDYFPEPVTVSWNSGALTSGVHTFPAVLQSSGLYSLSSVVTVPSSSLGTQTYICNVNHKPSNTKVDKRVEPKSCDKTH

SEQ ID NO: 56 - protein, 223 aa, Artificial; identical to SEQ ID NO: 37
  Chimeric homo sapiens mus musculus

SEQ ID NO: 57 - protein, 677 aa, Artificial
  Human-mouse chimeric
QVQLQQWGAGLLKPSETLSLTCAVYGGSFSGYYWSWIRQSPEKGLEWIGEINHGGYVTYNPSLESRVTISVDTSKNQFSLKLSSVTAADTAVYYCARDYGPGNYDWYFDLWGRGTLVTVSSASTKGPSVFPLAPSSKSTSGGTAALGCLVKDYFPEPVTVSWNSGALTSGVHTFPAVLQSSGLYSLSSVVTVPSSSLGTQTYICNVNHKPSNTKVDKRVEPKSCDKTHTCPPCPAPELLGGPSVFLFPPKPKDTLMISRTPEVTCVVVDVSHEDPEVKFNWYVDGVEVHNAKTKPREEQYNSTYRVVSVLTVLHQDWLNGKEYKCKVSNKALPAPIEKTISKAKGQPREPQVYTLPPSREEMTKNQVSLTCLVKGFYPSDIAVEWESNGQPENNYKTTPPVLDSDGSFFLYSKLTVDKSRWQQGNVFSCSVMHEALHNHYTQKSLSLSPGSTGSEVQLQQSGPELVKPGASVKISCKTSGYTFTEYTMHWVKQSHGKSLEWIGGISPNIGGTSYNQKFKGKATLTVDKSSSTAYMELRSLTSEDSAVYYCARRGGSFDYWGQGTTLTVSSRTVAAPSVFIFPPSDEQLKSGTASVVCLLNNFYPREAKVQWKVDNALQSGNSQESVTEQDSKDSTYSLSSTLTLSKADYEKHKVYACEVTHQGLSSPVTKSFNRGEC

SEQ ID NO: 58 - protein, 443 aa, Artificial
  Human-mouse chimeric
EIVLTQSPATLSLSPGERATLSCRASQSVSSYLAWYQQKPGQAPRLLIYDASNRATGIPARFSGSGSGTDFTLTISSLEPEDFAVYYCQQRSNWPPALTFCGGTKVEIKRTVAAPSVFIFPPSDEQLKSGTASVVCLLNNFYPREAKVQWKVDNALQSGNSQESVTEQDSKDSTYSLSSTLTLSKADYEKHKVYACEVTHQGLSSPVTKSFNRGECDKTHTCPPCPAPELLGGPSVFLFPPKPKDTLMISRTPEVTCVVVDVSHEDPEVKFNWYVDGVEVHNAKTKPREEQYNSTYRVVSVLTVLHQDWLNGKEYKCKVSNKALPAPIEKTISKAKGQPREPQVYTLPPSREEMTKNQVSLTCLVKGFYPSDIAVEWESNGQPENNYKTTPPVLDSDGSFFLYSKLTVDKSRWQQGNVFSCSVMHEALHNHYTQKSLSLSPGK

SEQ ID NO: 59 - protein, 469 aa, Artificial
  Human-mouse chimeric
DIVMTQSPATLSVTPGDRVSLSCRASQSISDYLHWYQQKSHESPRLLIKYASQSISGIPSRFSGSGSGSDFTLSINSVEPEDVGVYYCQNGHSFPLTFGAGTKLELKASTKGPSVFPLAPSSKSTSGGTAALGCLVKDYFPEPVTVSWNSGALTSGVHTFPAVLQSSGLYSLSSVVTVPSSSLGTQTYICNVNHKPSNTKVDKRVEPKSCDKTHGGSSSDIQLTQSPASLAVSLGQRATISCKASQSVDYDGDSYLNWYQQIPGQPPKLLIYDASNLVSGIPPRFSGSGSGTDFTLNIHPVEKVDAATYHCQQSTEDPWTFGGGTKLEIKGGGGSGGGGSGGGGSQVQLQQSGAELVRPGSSVKISCKASGYAFSSYWMNWVKQRPGQGLEWIGQIWPGDGDTNYNGKFKGKATLTADESSSTAYMQLSSLASEDSAVYFCARRETTTVGRYYYAMDYWGQGTTVTVSS

SEQ ID NO: 60 - protein, 680 aa, Artificial
  Human-mouse chimeric
QVQLVQSGAEVKKPGSSVKVSCKASGYAFSYSWINWVRQAPGQGLEWMGRIFPGDGDTDYNGKFKGRVTITADKSTSTAYMELSSLRSEDTAVYYCARNVFDGYWLVYWGQGTLVTVSSASTKGPSVFPLAPSSKSTSGGTAALGCLVKDYFPEPVTVSWNSGALTSGVHTFPAVLQSSGLYSLSSVVTVPSSSLGTQTYICNVNHKPSNTKVDKRVEPKSCDKTHTCPPCPAPELLGGPSVFLFPPKPKDTLMISRTPEVTCVVVDVSHEDPEVKFNWYVDGVEVHNAKTKPREEQYNSTYRVVSVLTVLHQDWLNGKEYKCKVSNKALPAPIEKTISKAKGQPREPQVYTLPPSREEMTKNQVSLTCLVKGFYPSDIAVEWESNGQPENNYKTTPPVLDSDGSFFLYSKLTVDKSRWQQGNVFSCSVMHEALHNHYTQKSLSLSPGSTGSQVQLQQPGAELVKPGASVKMSCKASGYTFTSYNMHWVKQTPGRGLEWIGAIYPGNGDTSYNQKFKGKATLTADKSSSTAYMQLSSLTSEDSAVYYCARSTYYGGDWYFNVWGAGTTVTVSARTVAAPSVFIFPPSDEQLKSGTASVVCLLNNFYPREAKVQWKVDNALQSGNSQESVTEQDSKDSTYSLSSTLTLSKADYEKHKVYACEVTHQGLSSPVTKSFNRGEC

SEQ ID NO: 61 - protein, 446 aa, Artificial
  Human-mouse chimeric
DIVMTQTPLSLPVTPGEPASISCRSSKSLLHSNGITYLYWYLQKPGQSPQLLIYQMSNLVSGVPDRFSGSGSGTDFTLKISRVEAEDVGVYYCAQNLELPYTFGGGTKVEIKRTVAAPSVFIFPPSDEQLKSGTASVVCLLNNFYPREAKVQWKVDNALQSGNSQESVTEQDSKDSTYSLSSTLTLSKADYEKHKVYACEVTHQGLSSPVTKSFNRGECDKTHTCPPCPAPELLGGPSVFLFPPKPKDTLMISRTPEVTCVVVDVSHEDPEVKFNWYVDGVEVHNAKTKPREEQYNSTYRVVSVLTVLHQDWLNGKEYKCKVSNKALPAPIEKTISKAKGQPREPQVYTLPPSREEMTKNQVSLTCLVKGFYPSDIAVEWESNGQPENNYKTTPPVLDSDGSFFLYSKLTVDKSRWQQGNVFSCSVMHEALHNHYTQKSLSLSPGK

SEQ ID NO: 62 - protein, 459 aa, Artificial
  Human-mouse chimeric
QIVLSQSPAILSASPGEKVTMTCRASSSVSYIHWFQQKPGSSPKPWIYATSNLASGVPVRFSGSGSGTSYSLTISRVEAEDAATYYCQQWTSNPPTFGGGTKLEIKASTKGPSVFPLAPSSKSTSGGTAALGCLVKDYFPEPVTVSWNSGALTSGVHTFPAVLQSSGLYSLSSVVTVPSSSLGTQTYICNVNHKPSNTKVDKRVEPKSCDKTHGGSSSEVQLQQSGPELVKPGASVKISCKTSGYTFTEYTMHWVKQSHGKSLEWIGGISPNIGGTSYNQKFKGKATLTVDKSSSTAYMELRSLTSEDSAVYYCARRGGSFDYWGQGTTLTVSSVEGGSGGSGGSGGSGGVDDIVMTQSPATLSVTPGDRVSLSCRASQSISDYLHWYQQKSHESPRLLIKYASQSISGIPSRFSGSGSGSDFTLSINSVEPEDVGVYYCQNGHSFPLTFGAGTKLELK

SEQ ID NO: 63 - protein, 443 aa, Artificial
  Human-mouse chimeric
EIVLTQSPATLSLSPGERATLSCRASQSVSSYLAWYQQKPGQAPRLLIYDASNRATGIPARFSGSGSGTDFTLTISSLEPEDFAVYYCQQRSNWPPALTFCGGTKVEIKRTVAAPSVFIFPPSDEQLKSGTASVVCLLNNFYPREAKVQWKVDNALQSGNSQESVTEQDSKDSTYSLSSTLTLSKADYEKHKVYACEVTHQGLSSPVTKSFNRGECDKTHTCPPCPAPELLGGPSVFLFPPKPKDTLMISRTPEVTCVVVDVSHEDPEVKFNWYVDGVEVHNAKTKPREEQYSSTYRVVSVLTVLHQDWLNGKEYKCKVSNKALPAPIEKTISKAKGQPREPQVYTLPPSREEMTKNQVSLTCLVKGFYPSDIAVEWESNGQPENNYKTTPPVLDSDGSFFLYSKLTVDKSRWQQGNVFSCSVMHEALHNHYTQKSLSLSPGK

SEQ ID NO: 64 - protein, 677 aa, Artificial
  Human-mouse chimeric
QVQLQQWGAGLLKPSETLSLTCAVYGGSFSGYYWSWIRQSPEKGLEWIGEINHGGYVTYNPSLESRVTISVDTSKNQFSLKLSSVTAADTAVYYCARDYGPGNYDWYFDLWGRGTLVTVSSASTKGPSVFPLAPSSKSTSGGTAALGCLVKDYFPEPVTVSWNSGALTSGVHTFPAVLQSSGLYSLSSVVTVPSSSLGTQTYICNVNHKPSNTKVDKRVEPKSCDKTHTCPPCPAPELLGGPSVFLFPPKPKDTLMISRTPEVTCVVVDVSHEDPEVKFNWYVDGVEVHNAKTKPREEQYSSTYRVVSVLTVLHQDWLNGKEYKCKVSNKALPAPIEKTISKAKGQPREPQVYTLPPSREEMTKNQVSLTCLVKGFYPSDIAVEWESNGQPENNYKTTPPVLDSDGSFFLYSKLTVDKSRWQQGNVFSCSVMHEALHNHYTQKSLSLSPGSTGSEVQLQQSGPELVKPGASVKISCKTSGYTFTEYTMHWVKQSHGKSLEWIGGISPNIGGTSYNQKFKGKATLTVDKSSSTAYMELRSLTSEDSAVYYCARRGGSFDYWGQGTTLTVSSRTVAAPSVFIFPPSDEQLKSGTASVVCLLNNFYPREAKVQWKVDNALQSGNSQESVTEQDSKDSTYSLSSTLTLSKADYEKHKVYACEVTHQGLSSPVTKSFNRGEC

SEQ ID NO: 65 - protein, 469 aa, Artificial; identical to SEQ ID NO: 59
  Human-mouse chimeric

SEQ ID NO: 66 - protein, 446 aa, Artificial
  Human-mouse chimeric
DIVMTQTPLSLPVTPGEPASISCRSSKSLLHSNGITYLYWYLQKPGQSPQLLIYQMSNLVSGVPDRFSGSGSGTDFTLKISRVEAEDVGVYYCAQNLELPYTFGGGTKVEIKRTVAAPSVFIFPPSDEQLKSGTASVVCLLNNFYPREAKVQWKVDNALQSGNSQESVTEQDSKDSTYSLSSTLTLSKADYEKHKVYACEVTHQGLSSPVTKSFNRGECDKTHTCPPCPAPELLGGPSVFLFPPKPKDTLMISRTPEVTCVVVDVSHEDPEVKFNWYVDGVEVHNAKTKPREEQYSSTYRVVSVLTVLHQDWLNGKEYKCKVSNKALPAPIEKTISKAKGQPREPQVYTLPPSREEMTKNQVSLTCLVKGFYPSDIAVEWESNGQPENNYKTTPPVLDSDGSFFLYSKLTVDKSRWQQGNVFSCSVMHEALHNHYTQKSLSLSPGK

SEQ ID NO: 67 - protein, 680 aa, Artificial
  Human-mouse chimeric
QVQLVQSGAEVKKPGSSVKVSCKASGYAFSYSWINWVRQAPGQGLEWMGRIFPGDGDTDYNGKFKGRVTITADKSTSTAYMELSSLRSEDTAVYYCARNVFDGYWLVYWGQGTLVTVSSASTKGPSVFPLAPSSKSTSGGTAALGCLVKDYFPEPVTVSWNSGALTSGVHTFPAVLQSSGLYSLSSVVTVPSSSLGTQTYICNVNHKPSNTKVDKRVEPKSCDKTHTCPPCPAPELLGGPSVFLFPPKPKDTLMISRTPEVTCVVVDVSHEDPEVKFNWYVDGVEVHNAKTKPREEQYSSTYRVVSVLTVLHQDWLNGKEYKCKVSNKALPAPIEKTISKAKGQPREPQVYTLPPSREEMTKNQVSLTCLVKGFYPSDIAVEWESNGQPENNYKTTPPVLDSDGSFFLYSKLTVDKSRWQQGNVFSCSVMHEALHNHYTQKSLSLSPGSTGSQVQLQQPGAELVKPGASVKMSCKASGYTFTSYNMHWVKQTPGRGLEWIGAIYPGNGDTSYNQKFKGKATLTADKSSSTAYMQLSSLTSEDSAVYYCARSTYYGGDWYFNVWGAGTTVTVSARTVAAPSVFIFPPSDEQLKSGTASVVCLLNNFYPREAKVQWKVDNALQSGNSQESVTEQDSKDSTYSLSSTLTLSKADYEKHKVYACEVTHQGLSSPVTKSFNRGEC

SEQ ID NO: 68 - protein, 459 aa, Artificial; identical to SEQ ID NO: 62
  Human-mouse chimeric

SEQ ID NO: 69 - protein, 216 aa, Artificial
  Human-mouse chimeric
EIVLTQSPATLSLSPGERATLSCRASQSVSSYLAWYQQKPGQAPRLLIYDASNRATGIPARFSGSGSGTDFTLTISSLEPEDFAVYYCQQRSNWPPALTFCGGTKVEIKRTVAAPSVFIFPPSDEQLKSGTASVVCLLNNFYPREAKVQWKVDNALQSGNSQESVTEQDSKDSTYSLSSTLTLSKADYEKHKVYACEVTHQGLSSPVTKSFNRGEC

SEQ ID NO: 70 - protein, 798 aa, Artificial
  Human-mouse chimeric
QVQLQQWGAGLLKPSETLSLTCAVYGGSFSGYYWSWIRQSPEKGLEWIGEINHGGYVTYNPSLESRVTISVDTSKNQFSLKLSSVTAADTAVYYCARDYGPGNYDWYFDLWGRGTLVTVSSASTKGPSVFPLAPSSKSTSGGTAALGCLVKDYFPEPVTVSWNSGALTSGVHTFPAVLQSSGLYSLSSVVTVPSSSLGTQTYICNVNHKPSNTKVDKRVEPKSCDKTHTSPPSPAPELLGGPSVFLFPPKPKDTLMISRTPEVTCVVVDVSHEDPEVKFNWYVDGVEVHNAKTKPREEQYSSTYRVVSVLTVLHQDWLNGKEYKCKVSNKALPAPIEKTISKAKGQPREPQVYTLPPSREEMTKNQVSLTCLVKGFYPSDIAVEWESNGQPENNYKTTPPVLDSDGSFFLYSKLTVDKSRWQQGNVFSCSVMHEALHNHYTQKSLSLSPGGGGGSGGGGSGGGGSGQPREPQVYTLPPSREEMTKNQVSLTCLVKGFYPSDIAVEWESNGQPENNYKTTPPVLDSDGSFFLYSKLTVDKSRWQQGNVFSCSVMHEALHNHYTQKSLSLSPGSTGSEVQLQQSGPELVKPGASVKISCKTSGYTFTEYTMHWVKQSHGKSLEWIGGISPNIGGTSYNQKFKGKATLTVDKSSSTAYMELRSLTSEDSAVYYCARRGGSFDYWGQGTTLTVSSRTVAAPSVFIFPPSDEQLKSGTASVVCLLNNFYPREAKVQWKVDNALQSGNSQESVTEQDSKDSTYSLSSTLTLSKADYEKHKVYACEVTHQGLSSPVTKSFNRGEC

SEQ ID NO: 71 - protein, 469 aa, Artificial; identical to SEQ ID NO: 59
  Human-mouse chimeric

SEQ ID NO: 72 - protein, 219 aa, Artificial
  Human-mouse chimeric
DIVMTQTPLSLPVTPGEPASISCRSSKSLLHSNGITYLYWYLQKPGQSPQLLIYQMSNLVSGVPDRFSGSGSGTDFTLKISRVEAEDVGVYYCAQNLELPYTFGGGTKVEIKRTVAAPSVFIFPPSDEQLKSGTASVVCLLNNFYPREAKVQWKVDNALQSGNSQESVTEQDSKDSTYSLSSTLTLSKADYEKHKVYACEVTHQGLSSPVTKSFNRGEC

SEQ ID NO: 73 - protein, 801 aa, Artificial
  Human-mouse chimeric
QVQLVQSGAEVKKPGSSVKVSCKASGYAFSYSWINWVRQAPGQGLEWMGRIFPGDGDTDYNGKFKGRVTITADKSTSTAYMELSSLRSEDTAVYYCARNVFDGYWLVYWGQGTLVTVSSASTKGPSVFPLAPSSKSTSGGTAALGCLVKDYFPEPVTVSWNSGALTSGVHTFPAVLQSSGLYSLSSVVTVPSSSLGTQTYICNVNHKPSNTKVDKRVEPKSCDKTHTSPPSPAPELLGGPSVFLFPPKPKDTLMISRTPEVTCVVVDVSHEDPEVKFNWYVDGVEVHNAKTKPREEQYSSTYRVVSVLTVLHQDWLNGKEYKCKVSNKALPAPIEKTISKAKGQPREPQVYTLPPSREEMTKNQVSLTCLVKGFYPSDIAVEWESNGQPENNYKTTPPVLDSDGSFFLYSKLTVDKSRWQQGNVFSCSVMHEALHNHYTQKSLSLSPGGGGGSGGGGSGGGGSGQPREPQVYTLPPSREEMTKNQVSLTCLVKGFYPSDIAVEWESNGQPENNYKTTPPVLDSDGSFFLYSKLTVDKSRWQQGNVFSCSVMHEALHNHYTQKSLSLSPGSTGSQVQLQQPGAELVKPGASVKMSCKASGYTFTSYNMHWVKQTPGRGLEWIGAIYPGNGDTSYNQKFKGKATLTADKSSSTAYMQLSSLTSEDSAVYYCARSTYYGGDWYFNVWGAGTTVTVSARTVAAPSVFIFPPSDEQLKSGTASVVCLLNNFYPREAKVQWKVDNALQSGNSQESVTEQDSKDSTYSLSSTLTLSKADYEKHKVYACEVTHQGLSSPVTKSFNRGEC

SEQ ID NO: 74 - protein, 459 aa, Artificial; identical to SEQ ID NO: 62
  Human-mouse chimeric

SEQ ID NO: 75 - protein, 814 aa, Artificial
  Human-mouse chimeric
EIVLTQSPATLSLSPGERATLSCRASQSVSSYLAWYQQKPGQAPRLLIYDASNRATGIPARFSGSGSGTDFTLTISSLEPEDFAVYYCQQRSNWPPALTFCGGTKVEIKGGGGSGGGGSGGGGSQVQLQQWGAGLLKPSETLSLTCAVYGGSFSGYYWSWIRQSPEKGLEWIGEINHGGYVTYNPSLESRVTISVDTSKNQFSLKLSSVTAADTAVYYCARDYGPGNYDWYFDLWGRGTLVTVSSGGGSSAPELLGGPSVFLFPPKPKDTLMISRTPEVTCVVVDVSHEDPEVKFNWYVDGVEVHNAKTKPREEQYSSTYRVVSVLTVLHQDWLNGKEYKCKVSNKALPAPIEKTISKAKGQPREPQVYTLPPSREEMTKNQVSLTCLVKGFYPSDIAVEWESNGQPENNYKTTPPVLDSDGSFFLYSKLTVDKSRWQQGNVFSCSVMHEALHNHYTQKSLSLSPGGGGGSGGGGSGGGGSGQPREPQVYTLPPSREEMTKNQVSLTCLVKGFYPSDIAVEWESNGQPENNYKTTPPVLDSDGSFFLYSKLTVDKSRWQQGNVFSCSVMHEALHNHYTQKSLSLSPGSTGSEVQLQQSGPELVKPGASVKISCKTSGYTFTEYTMHWVKQSHGKSLEWIGGISPNIGGTSYNQKFKGKATLTVDKSSSTAYMELRSLTSEDSAVYYCARRGGSFDYWGQGTTLTVSSRTVAAPSVFIFPPSDEQLKSGTASVVCLLNNFYPREAKVQWKVDNALQSGNSQESVTEQDSKDSTYSLSSTLTLSKADYEKHKVYACEVTHQGLSSPVTKSFNRGEC

SEQ ID NO: 76 - protein, 469 aa, Artificial; identical to SEQ ID NO: 59
  Human-mouse chimeric

SEQ ID NO: 77 - protein, 928 aa, Artificial
  Human-mouse chimeric
DIVMTQTPLSLPVTPGEPASISCRSSKSLLHSNGITYLYWYLQKPGQSPQLLIYQMSNLVSGVPDRFSGSGSGTDFTLKISRVEAEDVGVYYCAQNLELPYTFGGGTKVEIKGGGGSGGGGSGGGGSQVQLVQSGAEVKKPGSSVKVSCKASGYAFSYSWINWVRQAPGQGLEWMGRIFPGDGDTDYNGKFKGRVTITADKSTSTAYMELSSLRSEDTAVYYCARNVFDGYWLVYWGQGTLVTVSSASTKGPSVFPLAPSSKSTSGGTAALGCLVKDYFPEPVTVSWNSGALTSGVHTFPAVLQSSGLYSLSSVVTVPSSSLGTQTYICNVNHKPSNTKVDKRVEPKSCDKTHTSPPSPAPELLGGPSVFLFPPKPKDTLMISRTPEVTCVVVDVSHEDPEVKFNWYVDGVEVHNAKTKPREEQYSSTYRVVSVLTVLHQDWLNGKEYKCKVSNKALPAPIEKTISKAKGQPREPQVYTLPPSREEMTKNQVSLTCLVKGFYPSDIAVEWESNGQPENNYKTTPPVLDSDGSFFLYSKLTVDKSRWQQGNVFSCSVMHEALHNHYTQKSLSLSPGGGGGSGGGGSGGGGSGQPREPQVYTLPPSREEMTKNQVSLTCLVKGFYPSDIAVEWESNGQPENNYKTTPPVLDSDGSFFLYSKLTVDKSRWQQGNVFSCSVMHEALHNHYTQKSLSLSPGSTGSQVQLQQPGAELVKPGASVKMSCKASGYTFTSYNMHWVKQTPGRGLEWIGAIYPGNGDTSYNQKFKGKATLTADKSSSTAYMQLSSLTSEDSAVYYCARSTYYGGDWYFNVWGAGTTVTVSARTVAAPSVFIFPPSDEQLKSGTASVVCLLNNFYPREAKVQWKVDNALQSGNSQESVTEQDSKDSTYSLSSTLTLSKADYEKHKVYACEVTHQGLSSPVTKSFNRGEC

SEQ ID NO: 78 - protein, 459 aa, Artificial; identical to SEQ ID NO: 62
  Human-mouse chimeric